European Patent Application EP 4 603 597 A1, published August 20, 2025. Title: Age determination by determining DNA methylation levels of selected CpG sites. Applicant: Siemens Healthcare Diagnostics Products GmbH. Application EP. The sequence listing filed with the application follows.

SEQUENCE LISTING (22 sequences)

SEQ ID NO: 1 - DNA, 82 bp, Homo sapiens
  source 1..82: mol_type = genomic DNA
ggccgggcgggcttggggtgccctcctgcaaggtccccaccgacagcccccgagctctgcctcaggctgcaaatccggagcc

SEQ ID NO: 2 - DNA, 82 bp, Homo sapiens
  source 1..82: mol_type = genomic DNA
ccgcccgcgcttcccgacgctgccaggcaggctcccgggacgggcagagctccgaggctgcctccgggcagtcacgtccaac

SEQ ID NO: 3 - DNA, 82 bp, Homo sapiens
  source 1..82: mol_type = genomic DNA
tgggtctctcggaggagcaggagacgcgggctcgaagccgcgggcctgaccctgatccgtggatgccgccgccgccttctcc

SEQ ID NO: 4 - DNA, 82 bp, Homo sapiens
  source 1..82: mol_type = genomic DNA
gcggcggcgggggaggttgcgggggaggctcggcgtccccgctctccgccccgcgacaccgactgccgccgtggccgccctc

SEQ ID NO: 5 - DNA, 82 bp, Homo sapiens
  source 1..82: mol_type = genomic DNA
cggtggccgcgcgccgcccggctgttccgcgtccccttgccggctcacaatgtgctgaccctcccggccccgccgcgcgcct

SEQ ID NO: 6 - DNA, 82 bp, Homo sapiens
  source 1..82: mol_type = genomic DNA
cgccgctgggcgggcgcggcagggtcccggatccgtcctccgtgacgcgccggcttcctccggacactttccggcctctttt

SEQ ID NO: 7 - DNA, 82 bp, Homo sapiens
  source 1..82: mol_type = genomic DNA
gtggtggcgacagcggattccgtgcccggtggccgcgcgccgcccggctgttccgcgtccccttgccggctcacaatgtgct

SEQ ID NO: 8 - DNA, 82 bp, Homo sapiens
  source 1..82: mol_type = genomic DNA
gctgggcggcggccctgggctgctttggctaacttggctgcggggcaggcgcgaggagcggcgcgccgaccgggccgagcgg

SEQ ID NO: 9 - DNA, 82 bp, Homo sapiens
  source 1..82: mol_type = genomic DNA
ccggcgcgagctggagccgccaccggctgcctcggggtctcgccgggccttacctgctccgcgccctggaagcagatcttgc

SEQ ID NO: 10 - DNA, 82 bp, Homo sapiens
  source 1..82: mol_type = genomic DNA
actgccggagccctttgagcatcttctgcagagaatcgcccggagacccaagcctcagcagttctttggattaatgggcaaa

SEQ ID NO: 11 - DNA, 82 bp, Homo sapiens
  source 1..82: mol_type = genomic DNA
tagggagcgcgaatgggtctccgacagcaacgggagcagccggtggcgcctcaggctgcggtggcaacgagcccgactgcac

SEQ ID NO: 12 - DNA, 82 bp, Homo sapiens
  source 1..82: mol_type = genomic DNA
gcgcgcgctgcacatgaaggagcacccggattacaagtaccggccgcgccgcaagaccaagacgctgctcaagaaggacaag

SEQ ID NO: 13 - DNA, 82 bp, Homo sapiens
  source 1..82: mol_type = genomic DNA
tgcggtccatggcgcgacagtacaggtagcgctcggtgtccgagtagccgcgatgccggacgcggccggtggccccgctcga

SEQ ID NO: 14 - DNA, 82 bp, Homo sapiens
  source 1..82: mol_type = genomic DNA
ccccagtcccggtttccccgcggtgccggagcccggagctcgccgccgcccaggcctcaggaatcgagtaagtaacccctgt

SEQ ID NO: 15 - DNA, 82 bp, Homo sapiens
  source 1..82: mol_type = genomic DNA
ccgacctgcaggcgcgctaagcgctccgggcgccgcgctccgcgagggggagcagtgctcccaacccgcgaccctccgcctc

SEQ ID NO: 16 - DNA, 82 bp, Homo sapiens
  source 1..82: mol_type = genomic DNA
aggagctgcaggctcgggtccccagccaggcgggggactgcgggccgcccgcgctgcagggccgcgggtcaccgcagggggc

SEQ ID NO: 17 - DNA, 82 bp, Homo sapiens
  source 1..82: mol_type = genomic DNA
ggagagcgcggcggagtgagtgcggctgtggacccgggaccgggcgccgctgggcgggcgcggcagggtcccggatccgtcc

SEQ ID NO: 18 - DNA, 82 bp, Homo sapiens
  source 1..82: mol_type = genomic DNA
gcgaggcgctcattggccaatagggctgagtgacacgagtcggccccgagccgccctccgcgcgcccaggctccgggctctg

SEQ ID NO: 19 - DNA, 82 bp, Homo sapiens
  source 1..82: mol_type = genomic DNA
ggaccgcgggtgagcggtgggcaggtctcaggactctctccggacgtgcggtccggggccgcgccgggtgctgggcgcgcta

SEQ ID NO: 20 - DNA, 82 bp, Homo sapiens
  source 1..82: mol_type = genomic DNA
ctgcgtggtcgtcgtccaggatggtgacggtggccagcagcggcgccaccagccgccccttgggccgcccgccgccgtccgg

SEQ ID NO: 21 - DNA, 82 bp, Homo sapiens
  source 1..82: mol_type = genomic DNA
cagtgttcaggccccggggtttcccagccgtagtggccgccgccacagctgcgcgctttattgtctgctttcagtcgcaggt

SEQ ID NO: 22 - DNA, 82 bp, Homo sapiens
  source 1..82: mol_type = genomic DNA
ggagcgggaggcgtttcattggcggtggccgcagtggtggcggtggcggagagcgcggcggagtgagtgcggctgtggaccc